European Patent Application EP 4 706 646 A1, published March 11, 2026. Title: 一种新型的双链siRNA、其缀合物及其用途. Applicant: 广东东阳光药业股份有限公司. The sequence listing filed with the application follows.

SEQUENCE LISTING (46 sequences)

SEQ ID NO: 1 - RNA, 19 nt, Albies alba
  source 1..19: mol_type = other RNA
gygtgcacttcgcttcaca

SEQ ID NO: 2 - RNA, 19 nt, Albies alba
  source 1..19: mol_type = other RNA
gtytgcacttcgcttcaca

SEQ ID NO: 3 - RNA, 19 nt, Albies alba
  source 1..19: mol_type = other RNA
gtgygcacttcgcttcaca

SEQ ID NO: 4 - RNA, 19 nt, Albies alba
  source 1..19: mol_type = other RNA
gtgtycacttcgcttcaca

SEQ ID NO: 5 - RNA, 19 nt, Albies alba
  source 1..19: mol_type = other RNA
gtgtgyacttcgcttcaca

SEQ ID NO: 6 - RNA, 19 nt, Albies alba
  source 1..19: mol_type = other RNA
gtgtgcycttcgcttcaca

SEQ ID NO: 7 - RNA, 19 nt, Albies alba
  source 1..19: mol_type = other RNA
gtgtgcayttcgcttcaca

SEQ ID NO: 8 - RNA, 19 nt, Albies alba
  source 1..19: mol_type = other RNA
gtgtgcacytcgcttcaca

SEQ ID NO: 9 - RNA, 19 nt, Albies alba
  source 1..19: mol_type = other RNA
gtgtgcactycgcttcaca

SEQ ID NO: 10 - RNA, 19 nt, Albies alba
  source 1..19: mol_type = other RNA
gtgtgcacttygcttcaca

SEQ ID NO: 11 - RNA, 19 nt, Albies alba
  source 1..19: mol_type = other RNA
gtgtgcacttcycttcaca

SEQ ID NO: 12 - RNA, 19 nt, Albies alba
  source 1..19: mol_type = other RNA
gtgtgcacttcgyttcaca

SEQ ID NO: 13 - RNA, 19 nt, Albies alba
  source 1..19: mol_type = other RNA
gtgtgcacttcgcytcaca

SEQ ID NO: 14 - RNA, 19 nt, Albies alba
  source 1..19: mol_type = other RNA
gtgtgcacttcgctycaca

SEQ ID NO: 15 - RNA, 19 nt, Albies alba
  source 1..19: mol_type = other RNA
gtgtgcacttcgcttyaca

SEQ ID NO: 16 - RNA, 19 nt, Albies alba
  source 1..19: mol_type = other RNA
gtgtgcacttcgcttcyca

SEQ ID NO: 17 - RNA, 19 nt, Albies alba
  source 1..19: mol_type = other RNA
gtgtgcacttcgcttcaya

SEQ ID NO: 18 - RNA, 19 nt, Albies alba
  source 1..19: mol_type = other RNA
gtgtgcacttcgcttcacy

SEQ ID NO: 19 - RNA, 19 nt, Albies alba
  source 1..19: mol_type = other RNA
gtgtgcacttcgcttcaca

SEQ ID NO: 20 - RNA, 19 nt, Albies alba
  source 1..19: mol_type = other RNA
gtgtgcacttcgcttcaca

SEQ ID NO: 21 - RNA, 19 nt, Albies alba
  source 1..19: mol_type = other RNA
gtgtgcacttcgcttcyca

SEQ ID NO: 22 - RNA, 21 nt, Albies alba
  source 1..21: mol_type = other RNA
tytgaagcgaagtgcacactt

SEQ ID NO: 23 - RNA, 21 nt, Albies alba
  source 1..21: mol_type = other RNA
tgygaagcgaagtgcacactt

SEQ ID NO: 24 - RNA, 21 nt, Albies alba
  source 1..21: mol_type = other RNA
tgtyaagcgaagtgcacactt

SEQ ID NO: 25 - RNA, 21 nt, Albies alba
  source 1..21: mol_type = other RNA
tgtgyagcgaagtgcacactt

SEQ ID NO: 26 - RNA, 21 nt, Albies alba
  source 1..21: mol_type = other RNA
tgtgaygcgaagtgcacactt

SEQ ID NO: 27 - RNA, 21 nt, Albies alba
  source 1..21: mol_type = other RNA
tgtgaaycgaagtgcacactt

SEQ ID NO: 28 - RNA, 21 nt, Albies alba
  source 1..21: mol_type = other RNA
tgtgaagygaagtgcacactt

SEQ ID NO: 29 - RNA, 21 nt, Albies alba
  source 1..21: mol_type = other RNA
tgtgaagcgyagtgcacactt

SEQ ID NO: 30 - RNA, 21 nt, Albies alba
  source 1..21: mol_type = other RNA
tgtgaagcgaygtgcacactt

SEQ ID NO: 31 - RNA, 21 nt, Albies alba
  source 1..21: mol_type = other RNA
tgtgaagcgaagtgcycactt

SEQ ID NO: 32 - RNA, 21 nt, Albies alba
  source 1..21: mol_type = other RNA
tgtgaagcgaagtgcacyctt

SEQ ID NO: 33 - RNA, 21 nt, Albies alba
  source 1..21: mol_type = other RNA
tgtgaagcgaagtgcacactt

SEQ ID NO: 34 - RNA, 21 nt, Albies alba
  source 1..21: mol_type = other RNA
tgtgaagcgaagtgcycactt

SEQ ID NO: 35 - RNA, 21 nt, Albies alba
  source 1..21: mol_type = other RNA
tgtgaagcgaagtgcacyctt

SEQ ID NO: 36 - RNA, 21 nt, Albies alba
  source 1..21: mol_type = other RNA
tgtgaagcgaagtgcacactt

SEQ ID NO: 37 - RNA, 21 nt, Albies alba
  source 1..21: mol_type = other RNA
tgtgayycgaagtgcacactt

SEQ ID NO: 38 - RNA, 21 nt, Albies alba
  source 1..21: mol_type = other RNA
tgtgaagcgyagtgcacactt

SEQ ID NO: 39 - RNA, 21 nt, Albies alba
  source 1..21: mol_type = other RNA
tgtgaagcgaygtgcacactt

SEQ ID NO: 40 - RNA, 21 nt, Albies alba
  source 1..21: mol_type = other RNA
tgtgaagcgaagtgcacactt

SEQ ID NO: 41 - RNA, 19 nt, Albies alba
  source 1..19: mol_type = other RNA
gtgtgcacttcgcttyaca

SEQ ID NO: 42 - RNA, 19 nt, Albies alba
  source 1..19: mol_type = other RNA
gtgtgcacttcgcttcaca

SEQ ID NO: 43 - RNA, 19 nt, Albies alba
  source 1..19: mol_type = other RNA
gtgtgcacttcgcttcaca

SEQ ID NO: 44 - RNA, 19 nt, Albies alba
  source 1..19: mol_type = other RNA
gtgtgcacttcgcttcaya

SEQ ID NO: 45 - RNA, 19 nt, Albies alba
  source 1..19: mol_type = other RNA
gtgtgcacttcgcttcaca

SEQ ID NO: 46 - RNA, 21 nt, Albies alba
  source 1..21: mol_type = other RNA
tgtgaagcgaagtgcacactt